European Patent Application EP 4 356 923 A1, published April 24, 2024. Title: PKMYT1 FOR USE IN REGENERATIVE MEDICINE. Applicant: UNIVERSIDADE DE AVEIRO. Application EP. The sequence listing filed with the application follows.

SEQUENCE LISTING (12 sequences)

SEQ ID NO: 1 - DNA, 2247 bp, Synthetic construct
  source 1..2247: mol_type = other DNA
atggtgagcaagggcgaggagctgttcaccggggtggtgcccatcctggtcgagctggacggcgacgtaaacggccacaagttcagcgtgtccggcgagggcgagggcgatgccacctacggcaagctgaccctgaagttcatctgcaccaccggcaagctgcccgtgccctggcccaccctcgtgaccaccctgacctacggcgtgcagtgcttcagccgctaccccgaccacatgaagcagcacgacttcttcaagtccgccatgcccgaaggctacgtccaggagcgcaccatcttcttcaaggacgacggcaactacaagacccgcgccgaggtgaagttcgagggcgacaccctggtgaaccgcatcgagctgaagggcatcgacttcaaggaggacggcaacatcctggggcacaagctggagtacaactacaacagccacaacgtctatatcatggccgacaagcagaagaacggcatcaaggtgaacttcaagatccgccacaacatcgaggacggcagcgtgcagctcgccgaccactaccagcagaacacccccatcggcgacggccccgtgctgctgcccgacaaccactacctgagcacccagtccgccctgagcaaagaccccaacgagaagcgcgatcacatggtcctgctggagttcgtgaccgccgccgggatcactctcggcatggacgagctgtacaagtccggactcagatctcgagctcaagcttccatgctagaacggcctcctgcactggccatgcccatgcccacggagggcaccccgccacctctgagtggcacccccatcccagtcccagcctacttccgccacgcagaacctggattctccctcaagaggcccagggggctcagccggagcctcccacctccgccccctgccaagggcagcattcccatcagccgcctcttccctcctcggaccccaggctggcaccagctgcagccccggcgggtgtcattccggggcgaggcctcagagactctgcagagccctgggtatgacccaagccggccagagtccttcttccagcagagcttccagaggctcagccgcctgggccatggctcctacggagaggtcttcaaggtgcgctccaaggaggacggccggctctatgcggtaaagcgttccatgtcaccattccggggccccaaggaccgggcccgcaagttggccgaggtgggcagccacgagaaggtggggcagcacccatgctgcgtgcggctggagcaggcctgggaggagggcggcatcctgtacctgcagacggagctgtgcgggcccagcctgcagcaacactgtgaggcctggggtgccagcctgcctgaggcccaggtctggggctacctgcgggacacgctgcttgccctggcccatctgcacagccagggcctggtgcaccttgatgtcaagcctgccaacatcttcctggggccccggggccgctgcaagctgggtgacttcggactgctggtggagctgggtacagcaggagctggtgaggtccaggagggagacccccgctacatggcccccgagctgctgcagggctcctatgggacagcagcggatgtgttcagtctgggcctcaccatcctggaagtggcatgcaacatggagctgccccacggtggggagggctggcagcagctgcgccagggctacctgccccctgagttcactgccggtctgtcttccgagctgcgttctgtccttgtcatgatgctggagccagaccccaagctgcgggccacggccgaggccctgctggcactgcctgtgttgaggcagccgcgggcctggggtgtgctgtggtgcatggcagcggaggccctgagccgagggtgggccctgtggcaggccctgcttgccctgctctgctggctctggcatgggctggctcaccctgccagctggctacagcccctgggcccgccagccaccccgcctggctcaccaccctgcagtttgctcctggacagcagcctctccagcaactgggatgacgacagcctagggccttcactctcccctgaggctgtcctggcccggactgtggggagcacctccaccccccggagcaggtgcacacccagggatgccctggacctaagtgacatcaactcagagcctcctcggggctccttcccctcctttgagcctcggaacctcctcagcctgtttgaggacaccctagacccaacctga

SEQ ID NO: 2 - RNA, 21 nt, Synthetic construct
  source 1..21: mol_type = other RNA
  modified_base 20..21: mod_base = OTHER; note = thymine
gtggcatgcaacatggagctt

SEQ ID NO: 3 - RNA, 21 nt, Synthetic construct
  source 1..21: mol_type = other RNA
  modified_base 20..21: mod_base = OTHER; note = thymine
gctccatgttgcatgccactt

SEQ ID NO: 4 - DNA, 29 bp, Synthetic construct
  source 1..29: mol_type = other DNA
aataagcttccatgctagaacggcctcct

SEQ ID NO: 5 - DNA, 27 bp, Synthetic construct
  source 1..27: mol_type = other DNA
ataggatcctcaggttgggtctagggt

SEQ ID NO: 6 - DNA, 2061 bp, Homo sapiens
  source 1..2061: mol_type = genomic DNA
gcgcgttcacgggccgttccccctcacgggagtcctccgcccgggcgtccggaacagtcgacggcagactccggcccgctgagccacccgaggggtcccgtggcctccgcggacccggaatctgggccctcgcggacccgcgccccgcccagtcgccccagggcttccccacacccacggagtgaagtcagccgcggccctgcctgggaggaacttaccgtctaccgggaaaggtggccagcagatgtgtcgggcctggtgagagggtgaggcgagacggcccgatcgcccagggccccggaagctgcggaggtcacccccgcctggccttagctcagggacaccctggattcacgtgggagcccctgctcctgcctcccccgtcccaccactgaggctgttgggccaggccagtcatgctagaacggcctcctgcactggccatgcccatgcccacggagggcaccccgccacctctgagtggcacccccatcccagtcccagcctacttccgccacgcagaacctggattctccctcaagaggcccagggggctcagccggagcctcccacctccgccccctgccaagggcagcattcccatcagccgcctcttccctcctcggaccccaggctggcaccagctgcagccccggcgggtgtcattccggggcgaggcctcagagactctgcagagccctgggtatgacccaagccggccagagtccttcttccagcagagcttccagaggctcagccgcctgggccatggctcctacggagaggtcttcaaggtgcgctccaaggaggacggccggctctatgcggtaaagcgttccatgtcaccattccggggccccaaggaccgggcccgcaagttggccgaggtgggcagccacgagaaggtggggcagcacccatgctgcgtgcggctggagcaggcctgggaggagggcggcatcctgtacctgcagacggagctgtgcgggcccagcctgcagcaacactgtgaggcctggggtgccagcctgcctgaggcccaggtctggggctacctgcgggacacgctgcttgccctggcccatctgcacagccagggcctggtgcaccttgatgtcaagcctgccaacatcttcctggggccccggggccgctgcaagctgggtgacttcggactgctggtggagctgggtacagcaggagctggtgaggtccaggagggagacccccgctacatggcccccgagctgctgcagggctcctatgggacagcagcggatgtgttcagtctgggcctcaccatcctggaagtggcatgcaacatggagctgccccacggtggggagggctggcagcagctgcgccagggctacctgccccctgagttcactgccggtctgtcttccgagctgcgttctgtccttgtcatgatgctggagccagaccccaagctgcgggccacggccgaggccctgctggcactgcctgtgttgaggcagccgcgggcctggggtgtgctgtggtgcatggcagcggaggccctgagccgagggtgggccctgtggcaggccctgcttgccctgctctgctggctctggcatgggctggctcaccctgccagctggctacagcccctgggcccgccagccaccccgcctggctcaccaccctgcagtttgctcctggacagcagcctctccagcaactgggatgacgacagcctagggccttcactctcccctgaggctgtcctggcccggactgtggggagcacctccaccccccggagcaggtgcacacccagggatgccctggacctaagtgacatcaactcagagcctcctcggggctccttcccctcctttgagcctcggaacctcctcagcctgtttgaggacaccctagacccaacctgagccccagactctgcctctgcacttttaaccttttatcctgtgtctctcccgtcgcccttgaaagctggggcccctcgggaactcccatggtcttctctgcctggccgtgtctaataaaaagtatttgaaccttgggagcacccaa

SEQ ID NO: 7 - DNA, 1500 bp, Homo sapiens
  source 1..1500: mol_type = genomic DNA
atgctagaacggcctcctgcactggccatgcccatgcccacggagggcaccccgccacctctgagtggcacccccatcccagtcccagcctacttccgccacgcagaacctggattctccctcaagaggcccagggggctcagccggagcctcccacctccgccccctgccaagggcagcattcccatcagccgcctcttccctcctcggaccccaggctggcaccagctgcagccccggcgggtgtcattccggggcgaggcctcagagactctgcagagccctgggtatgacccaagccggccagagtccttcttccagcagagcttccagaggctcagccgcctgggccatggctcctacggagaggtcttcaaggtgcgctccaaggaggacggccggctctatgcggtaaagcgttccatgtcaccattccggggccccaaggaccgggcccgcaagttggccgaggtgggcagccacgagaaggtggggcagcacccatgctgcgtgcggctggagcaggcctgggaggagggcggcatcctgtacctgcagacggagctgtgcgggcccagcctgcagcaacactgtgaggcctggggtgccagcctgcctgaggcccaggtctggggctacctgcgggacacgctgcttgccctggcccatctgcacagccagggcctggtgcaccttgatgtcaagcctgccaacatcttcctggggccccggggccgctgcaagctgggtgacttcggactgctggtggagctgggtacagcaggagctggtgaggtccaggagggagacccccgctacatggcccccgagctgctgcagggctcctatgggacagcagcggatgtgttcagtctgggcctcaccatcctggaagtggcatgcaacatggagctgccccacggtggggagggctggcagcagctgcgccagggctacctgccccctgagttcactgccggtctgtcttccgagctgcgttctgtccttgtcatgatgctggagccagaccccaagctgcgggccacggccgaggccctgctggcactgcctgtgttgaggcagccgcgggcctggggtgtgctgtggtgcatggcagcggaggccctgagccgagggtgggccctgtggcaggccctgcttgccctgctctgctggctctggcatgggctggctcaccctgccagctggctacagcccctgggcccgccagccaccccgcctggctcaccaccctgcagtttgctcctggacagcagcctctccagcaactgggatgacgacagcctagggccttcactctcccctgaggctgtcctggcccggactgtggggagcacctccaccccccggagcaggtgcacacccagggatgccctggacctaagtgacatcaactcagagcctcctcggggctccttcccctcctttgagcctcggaacctcctcagcctgtttgaggacaccctagacccaacctga

SEQ ID NO: 8 - protein, 499 aa, Homo sapiens
MLERPPALAMPMPTEGTPPPLSGTPIPVPAYFRHAEPGFSLKRPRGLSRSLPPPPPAKGSIPISRLFPPRTPGWHQLQPRRVSFRGEASETLQSPGYDPSRPESFFQQSFQRLSRLGHGSYGEVFKVRSKEDGRLYAVKRSMSPFRGPKDRARKLAEVGSHEKVGQHPCCVRLEQAWEEGGILYLQTELCGPSLQQHCEAWGASLPEAQVWGYLRDTLLALAHLHSQGLVHLDVKPANIFLGPRGRCKLGDFGLLVELGTAGAGEVQEGDPRYMAPELLQGSYGTAADVFSLGLTILEVACNMELPHGGEGWQQLRQGYLPPEFTAGLSSELRSVLVMMLEPDPKLRATAEALLALPVLRQPRAWGVLWCMAAEALSRGWALWQALLALLCWLWHGLAHPASWLQPLGPPATPPGSPPCSLLLDSSLSSNWDDDSLGPSLSPEAVLARTVGSTSTPRSRCTPRDALDLSDINSEPPRGSFPSFEPRNLLSLFEDTLDPT

SEQ ID NO: 9 - protein, 480 aa, Homo sapiens
MLERPPALAMPMPTEGTPPPLSGTPIPVPAYFRHAEPGFSLKRPRGLSRSLPPPPPAKGSIPISRLFPPRTPGWHQLQPRRVSFRGEASETLQSPGYDPSRPESFFQQSFQRLSRLGHGSYGEVFKVRSKEDGRLYAVKRSMSPFRGPKDRARKLAEVGSHEKVGQHPCCVRLEQAWEEGGILYLQTELCGPSLQQHCEAWGASLPEAQVWGYLRDTLLALAHLHSQGLVHLDVKPANIFLGPRGRCKLGDFGLLVELGTAGAGEVQEGDPRYMAPELLQGSYGTAADVFSLGLTILEVACNMELPHGGEGWQQLRQGYLPPEFTAGLSSELRSVLVMMLEPDPKLRATAEALLALPVLRQPRAWGVLWCMAAEALSRGWALWQALLALLCWLWHGLAHPASWLQPLGPPATPPGSPPCSLLLDSSLSSNWDDDSLGPGHPPCLACPPAGLHSPLRLSWPGLWGAPPPPGAGAHPGMPWT

SEQ ID NO: 10 - protein, 490 aa, Homo sapiens
MPMPTEGTPPPLSGTPIPVPAYFRHAEPGFSLKRPRGLSRSLPPPPPAKGSIPISRLFPPRTPGWHQLQPRRVSFRGEASETLQSPGYDPSRPESFFQQSFQRLSRLGHGSYGEVFKVRSKEDGRLYAVKRSMSPFRGPKDRARKLAEVGSHEKVGQHPCCVRLEQAWEEGGILYLQTELCGPSLQQHCEAWGASLPEAQVWGYLRDTLLALAHLHSQGLVHLDVKPANIFLGPRGRCKLGDFGLLVELGTAGAGEVQEGDPRYMAPELLQGSYGTAADVFSLGLTILEVACNMELPHGGEGWQQLRQGYLPPEFTAGLSSELRSVLVMMLEPDPKLRATAEALLALPVLRQPRAWGVLWCMAAEALSRGWALWQALLALLCWLWHGLAHPASWLQPLGPPATPPGSPPCSLLLDSSLSSNWDDDSLGPSLSPEAVLARTVGSTSTPRSRCTPRDALDLSDINSEPPRGSFPSFEPRNLLSLFEDTLDPT

SEQ ID NO: 11 - protein, 430 aa, Homo sapiens
MLERWHQLQPRRVSFRGEASETLQSPGYDPSRPESFFQQSFQRLSRLGHGSYGEVFKVRSKEDGRLYAVKRSMSPFRGPKDRARKLAEVGSHEKVGQHPCCVRLEQAWEEGGILYLQTELCGPSLQQHCEAWGASLPEAQVWGYLRDTLLALAHLHSQGLVHLDVKPANIFLGPRGRCKLGDFGLLVELGTAGAGEVQEGDPRYMAPELLQGSYGTAADVFSLGLTILEVACNMELPHGGEGWQQLRQGYLPPEFTAGLSSELRSVLVMMLEPDPKLRATAEALLALPVLRQPRAWGVLWCMAAEALSRGWALWQALLALLCWLWHGLAHPASWLQPLGPPATPPGSPPCSLLLDSSLSSNWDDDSLGPSLSPEAVLARTVGSTSTPRSRCTPRDALDLSDINSEPPRGSFPSFEPRNLLSLFEDTLDPT

SEQ ID NO: 12 - DNA, 747 bp, synthetic construct
  source 1..747: mol_type = other DNA
atggtgagcaagggcgaggagctgttcaccggggtggtgcccatcctggtcgagctggacggcgacgtaaacggccacaagttcagcgtgtccggcgagggcgagggcgatgccacctacggcaagctgaccctgaagttcatctgcaccaccggcaagctgcccgtgccctggcccaccctcgtgaccaccctgacctacggcgtgcagtgcttcagccgctaccccgaccacatgaagcagcacgacttcttcaagtccgccatgcccgaaggctacgtccaggagcgcaccatcttcttcaaggacgacggcaactacaagacccgcgccgaggtgaagttcgagggcgacaccctggtgaaccgcatcgagctgaagggcatcgacttcaaggaggacggcaacatcctggggcacaagctggagtacaactacaacagccacaacgtctatatcatggccgacaagcagaagaacggcatcaaggtgaacttcaagatccgccacaacatcgaggacggcagcgtgcagctcgccgaccactaccagcagaacacccccatcggcgacggccccgtgctgctgcccgacaaccactacctgagcacccagtccgccctgagcaaagaccccaacgagaagcgcgatcacatggtcctgctggagttcgtgaccgccgccgggatcactctcggcatggacgagctgtacaagtccggactcagatctcgagctcaagcttcc